European Patent Specification EP 4 146 817 B1, published August 5, 2026. Title: LIQUID BIOPSY PLATFORM IN PLASMA AND SALIVA. Applicant: The Regents of the University of California Wong, David Wei, Fang Strom, Charles Tu, Michael Liao, Wei Cheng, Jordan Chia, David Tang, Hieu Ye, Qianlin Li, Feng. The sequence listing filed with the application follows.

SEQUENCE LISTING (15 sequences)

SEQ ID NO: 1 - DNA, 85 bp, Artificial Sequence
  Chemcially synthesized,
aaaaaaaaaagaaataaacaaataaaacaataacaaataaaaaaaaacaaataaacaataaaaaaaaacaagtttgacccgccca

SEQ ID NO: 2 - DNA, 39 bp, Artificial Sequence
  Chemcially synthesized, L858R Detector Probe
aaaatctgtgatcttgacatgctgcggtgttttgtgcag

SEQ ID NO: 3 - DNA, 54 bp, Artificial Sequence
  Chemcially synthesized, Control calibrator oligo L858R wild type
ctggtgaaaacaccgcagcatgtcaagatcacagattttgggctggccaaactg

SEQ ID NO: 4 - DNA, 54 bp, Artificial Sequence
  Chemcially synthesized, control calibrator oligo L858R mutant
ctggtgaaaacaccgcagcatgtcaagatcacagattttgggcgggccaaactg

SEQ ID NO: 5 - DNA, 80 bp, Artificial Sequence
  Chemcially synthesized, Exon19 del Capture Probe
aaaaaaaaaaaaataaaaaaaaaaaaataaaaaaaaaaaaataaaaaaaaaaaaataaaaaaaaacatgttgcttccttg

SEQ ID NO: 6 - DNA, 30 bp, Artificial Sequence
  Chemcially synthesized, Exon19 del Detector Probe
atagcgacgggaattttaactttctcacct

SEQ ID NO: 7 - DNA, 57 bp, Artificial Sequence
  Chemcially synthesized, Control calibrator oligo Exon19 Mutation Del
aggtgagaaagttaaaattcccgtcgctatcaaggaagcaacatctccgaaagccaa

SEQ ID NO: 8 - DNA, 65 bp, Artificial Sequence
  Chemcially synthesized, Control calibrator oligo Exon19 del Wild type
aggtgagaaagttaaaattcccgtcgctatcaaggaattaagagaagcaacatctccgaaagcca

SEQ ID NO: 9 - DNA, 85 bp, Artificial Sequence
  Chemcially synthesized, T790M Capture Probe
aaaaaaaaaagaaataaacaaataaaacaataacaaataaaaaaaaacaaataaacaataaaaaaaaacaagagcggcatgatga

SEQ ID NO: 10 - DNA, 32 bp, Artificial Sequence
  Chemcially synthesized, T790M Detector Probe
gctgcacggtggaggtgaggcagatgcccagc

SEQ ID NO: 11 - DNA, 52 bp, Artificial Sequence
  Chemcially synthesized, Control calibrator oligo T790M
gctgggcatctgcctcacctccaccgtgcagctcatcatgcagctcatgccc

SEQ ID NO: 12 - DNA, 52 bp, Artificial Sequence
  Chemcially synthesized, Control calibrator oligo T790M Wildtype Sequence
gctgggcatctgcctcacctccaccgtgcagctcatcacgcagctcatgccc

SEQ ID NO: 13 - DNA, 13 bp, Artificial Sequence
  Chemcially synthesized, Exon 19del capture probe
tgttgcttccttg

SEQ ID NO: 14 - DNA, 14 bp, Artificial Sequence
  Chemcially synthesized, p.L858R capture probe
gtttgacccgccca

SEQ ID NO: 15 - DNA, 14 bp, Artificial Sequence
  Chemcially synthesized, p,T790M Capture Probe
gagcggcatgatga